European Patent Application EP 4 678 003 A1, published January 14, 2026. Title: METHODS AND COMPOSITIONS FOR THE CONTROL IN THE FIELD OF INFECTIOUS DISEASES IN PLANTS. Applicant: UNIVERSITAT DE GIRONA. Application EP. The sequence listing filed with the application follows.

SEQUENCE LISTING (24 sequences)

SEQ ID NO: 1 - protein, 22 aa, Prunus persica
EVAASSRVVRQPITTGGGGQIN

SEQ ID NO: 2 - protein, 23 aa, Prunus persica
YVQRITLRAARPEISTGSGAQTN

SEQ ID NO: 3 - protein, 248 aa, synthetic construct
MSPILGYWKIKGLVQPTRLLLEYLEEKYEEHLYERDEGDKWRNKKFELGLEFPNLPYYIDGDVKLTQSMAIIRYIADKHNMLGGCPKERAEISMLEGAVLDIRYGVSRIAYSKDFETLKVDFLSKLPEMLKMFEDRLCHKTYLNGDHVTHPDFMLYDALDVVLYMDPMCLDAFPKLVCFKKRIEAIPQIDKYLKSSKYIAWPLQGWQATFGGGDHPPKSDLVPRGSEVAASSRVVRQPITTGGGGQIN

SEQ ID NO: 4 - protein, 249 aa, synthetic construct
MSPILGYWKIKGLVQPTRLLLEYLEEKYEEHLYERDEGDKWRNKKFELGLEFPNLPYYIDGDVKLTQSMAIIRYIADKHNMLGGCPKERAEISMLEGAVLDIRYGVSRIAYSKDFETLKVDFLSKLPEMLKMFEDRLCHKTYLNGDHVTHPDFMLYDALDVVLYMDPMCLDAFPKLVCFKKRIEAIPQIDKYLKSSKYIAWPLQGWQATFGGGDHPPKSDLVPRGSYVQRITLRAARPEISTGSGAQTN

SEQ ID NO: 5 - protein, 23 aa, synthetic construct
XXXXXXXRXXRXXJXXGXGXQXN

SEQ ID NO: 6 - protein, 28 aa, synthetic construct
XXXAXYXRIXXXXXEXPXXSXGXGGXXX

SEQ ID NO: 7 - protein, 23 aa, Solanum lycopersicum
ATDRRGRPPSRPKVGSGPPPQNN

SEQ ID NO: 8 - protein, 249 aa, synthetic construct
MSPILGYWKIKGLVQPTRLLLEYLEEKYEEHLYERDEGDKWRNKKFELGLEFPNLPYYIDGDVKLTQSMAIIRYIADKHNMLGGCPKERAEISMLEGAVLDIRYGVSRIAYSKDFETLKVDFLSKLPEMLKMFEDRLCHKTYLNGDHVTHPDFMLYDALDVVLYMDPMCLDAFPKLVCFKKRIEAIPQIDKYLKSSKYIAWPLQGWQATFGGGDHPPKSDLVPRGSATDRRGRPPSRPKVGSGPPPQNN

SEQ ID NO: 9 - protein, 32 aa, Fragaria X ananassa
EDVVVVATGTARSTRALGVKRPIGTGSGPQIN

SEQ ID NO: 10 - protein, 32 aa, Fragaria X ananassa
EEGVVIATGTARSTRALRMKRSIGSGSGPQIN

SEQ ID NO: 11 - protein, 32 aa, Fragaria vesca; identical to SEQ ID NO: 9

SEQ ID NO: 12 - protein, 21 aa, Malus domestica
QRGIVCAENPPLSTGSGGQIN

SEQ ID NO: 13 - protein, 28 aa, Malus domestica
DEAAEVTRIKVSTRERPGLSTGEGGKTN

SEQ ID NO: 14 - protein, 22 aa, Prunus avium
EVAVSFRVVRPPITRGGGGQIN

SEQ ID NO: 15 - protein, 23 aa, Prunus avium
YVQRITLRAARPELSTGGGAQTN

SEQ ID NO: 16 - protein, 22 aa, Prunus dulcis
EVAASSRVIRPPITTGEGGQIN

SEQ ID NO: 17 - protein, 23 aa, Prunus dulcis
YVQRITLRAARPEISTGSGAQTN

SEQ ID NO: 18 - protein, 22 aa, Prunus domestica
EVAGSLRAVRPPITTGGGGQIN

SEQ ID NO: 19 - protein, 23 aa, Prunus domestica
YVQRITLRAARPEISTGSGAQTN

SEQ ID NO: 20 - protein, 22 aa, Prunus mume
EVAGSLRAVRPPITTGGGGQIN

SEQ ID NO: 21 - protein, 23 aa, Prunus mume
YVQRITLRAARPEISTGSGAQTN

SEQ ID NO: 22 - protein, 22 aa, Prunus nucipersica
EVAASSRVVRQPITTGGGGQIN

SEQ ID NO: 23 - protein, 23 aa, Prunus nucipersica
YVQRITLRAARPEISTGSGAQTN

SEQ ID NO: 24 - protein, 28 aa, Pyrus bretschneideri
DEAAAITRIKVSARERPGLSTGKGGKTN